European Patent Application EP 4 656 651 A1, published December 3, 2025. Title: A microorganism having Threonine/homoserine exporter variant and a method for producing L-amino acid using the same. Applicant: CJ CheilJedang Corporation. The sequence listing filed with the application follows.

SEQUENCE LISTING (122 sequences)

SEQ ID NO: 1 - protein, 295 aa, Escherichia coli
  source 1..295: note = RhtA WT AA
MPGSLRKMPVWLPIVILLVAMASIQGGASLAKSLFPLVGAPGVTALRLALGTLILIAFFKPWRLRFAKEQRLPLLFYGVSLGGMNYLFYLSIQTVPLGIAVALEFTGPLAVALFSSRRPVDFVWVVLAVLGLWFLLPLGQDVSHVDLTGCALALGAGACWAIYILSGQRAGAEHGPATVAIGSLIAALIFVPIGALQAGEALWHWSVIPLGLAVAILSTALPYSLEMIALTRLPTRTFGTLMSMEPALAAVSGMIFLGETLTPIQLLALGAIIAASMGSTLTVRKESKIKELDIN

SEQ ID NO: 2 - DNA, 888 bp, Escherichia coli
  source 1..888: mol_type = genomic DNA; note = RhtA WT NT
atgcctggttcattacgtaaaatgccggtctggttaccaatagtcatattgctcgttgccatggcgtctattcagggtggagcctcgttagctaagtcactttttcctctggtgggcgcaccgggtgtcactgcgctgcgtctggcattaggaacgctgatcctcatcgcgttctttaagccatggcgactgcgctttgccaaagagcaacggttaccgctgttgttttacggcgtttcgctgggtgggatgaattatcttttttatctttctattcagacagtaccgctgggtattgcggtggcgctggagttcaccggaccactggcggtggcgctgttctcttctcgtcgcccggtagatttcgtctgggttgtgctggcggttcttggtctgtggttcctgctaccgctggggcaagacgtttcccatgtcgatttaaccggctgtgcgctggcactgggggccggggcttgttgggctatttacattttaagtgggcaacgcgcaggagcggaacatggccctgcgacggtggcaattggttcgttgattgcagcgttaattttcgtgccaattggagcgcttcaggctggtgaagcactctggcactggtcggttattccattgggtctggctgtcgctattctctcgaccgctctgccttattcgctggaaatgattgccctcacccgtttgccaacacggacatttggtacgctgatgagcatggaaccggcgctggctgccgtttccgggatgattttcctcggagaaacactgacacccatacagctactggcgctcggcgctatcatcgccgcttcaatggggtctacgctgacagtacgcaaagagagcaaaataaaagaattagacattaattaa

SEQ ID NO: 3 - protein, 295 aa, synthetic construct
  source 1..295: note = RhtA V123A AA
MPGSLRKMPVWLPIVILLVAMASIQGGASLAKSLFPLVGAPGVTALRLALGTLILIAFFKPWRLRFAKEQRLPLLFYGVSLGGMNYLFYLSIQTVPLGIAVALEFTGPLAVALFSSRRPVDFAWVVLAVLGLWFLLPLGQDVSHVDLTGCALALGAGACWAIYILSGQRAGAEHGPATVAIGSLIAALIFVPIGALQAGEALWHWSVIPLGLAVAILSTALPYSLEMIALTRLPTRTFGTLMSMEPALAAVSGMIFLGETLTPIQLLALGAIIAASMGSTLTVRKESKIKELDIN

SEQ ID NO: 4 - DNA, 888 bp, synthetic construct
  source 1..888: mol_type = other DNA; note = RhtA V123A NT
atgcctggttcattacgtaaaatgccggtctggttaccaatagtcatattgctcgttgccatggcgtctattcagggtggagcctcgttagctaagtcactttttcctctggtgggcgcaccgggtgtcactgcgctgcgtctggcattaggaacgctgatcctcatcgcgttctttaagccatggcgactgcgctttgccaaagagcaacggttaccgctgttgttttacggcgtttcgctgggtgggatgaattatcttttttatctttctattcagacagtaccgctgggtattgcggtggcgctggagttcaccggaccactggcggtggcgctgttctcttctcgtcgcccggtagatttcgcctgggttgtgctggcggttcttggtctgtggttcctgctaccgctggggcaagacgtttcccatgtcgatttaaccggctgtgcgctggcactgggggccggggcttgttgggctatttacattttaagtgggcaacgcgcaggagcggaacatggccctgcgacggtggcaattggttcgttgattgcagcgttaattttcgtgccaattggagcgcttcaggctggtgaagcactctggcactggtcggttattccattgggtctggctgtcgctattctctcgaccgctctgccttattcgctggaaatgattgccctcacccgtttgccaacacggacatttggtacgctgatgagcatggaaccggcgctggctgccgtttccgggatgattttcctcggagaaacactgacacccatacagctactggcgctcggcgctatcatcgccgcttcaatggggtctacgctgacagtacgcaaagagagcaaaataaaagaattagacattaattaa

SEQ ID NO: 5 - protein, 295 aa, synthetic construct
  source 1..295: note = RhtA V123C AA
MPGSLRKMPVWLPIVILLVAMASIQGGASLAKSLFPLVGAPGVTALRLALGTLILIAFFKPWRLRFAKEQRLPLLFYGVSLGGMNYLFYLSIQTVPLGIAVALEFTGPLAVALFSSRRPVDFCWVVLAVLGLWFLLPLGQDVSHVDLTGCALALGAGACWAIYILSGQRAGAEHGPATVAIGSLIAALIFVPIGALQAGEALWHWSVIPLGLAVAILSTALPYSLEMIALTRLPTRTFGTLMSMEPALAAVSGMIFLGETLTPIQLLALGAIIAASMGSTLTVRKESKIKELDIN

SEQ ID NO: 6 - DNA, 888 bp, synthetic construct
  source 1..888: mol_type = other DNA; note = RhtA V123C NT
atgcctggttcattacgtaaaatgccggtctggttaccaatagtcatattgctcgttgccatggcgtctattcagggtggagcctcgttagctaagtcactttttcctctggtgggcgcaccgggtgtcactgcgctgcgtctggcattaggaacgctgatcctcatcgcgttctttaagccatggcgactgcgctttgccaaagagcaacggttaccgctgttgttttacggcgtttcgctgggtgggatgaattatcttttttatctttctattcagacagtaccgctgggtattgcggtggcgctggagttcaccggaccactggcggtggcgctgttctcttctcgtcgcccggtagatttctgctgggttgtgctggcggttcttggtctgtggttcctgctaccgctggggcaagacgtttcccatgtcgatttaaccggctgtgcgctggcactgggggccggggcttgttgggctatttacattttaagtgggcaacgcgcaggagcggaacatggccctgcgacggtggcaattggttcgttgattgcagcgttaattttcgtgccaattggagcgcttcaggctggtgaagcactctggcactggtcggttattccattgggtctggctgtcgctattctctcgaccgctctgccttattcgctggaaatgattgccctcacccgtttgccaacacggacatttggtacgctgatgagcatggaaccggcgctggctgccgtttccgggatgattttcctcggagaaacactgacacccatacagctactggcgctcggcgctatcatcgccgcttcaatggggtctacgctgacagtacgcaaagagagcaaaataaaagaattagacattaattaa

SEQ ID NO: 7 - protein, 295 aa, synthetic construct
  source 1..295: note = RhtA V123D AA
MPGSLRKMPVWLPIVILLVAMASIQGGASLAKSLFPLVGAPGVTALRLALGTLILIAFFKPWRLRFAKEQRLPLLFYGVSLGGMNYLFYLSIQTVPLGIAVALEFTGPLAVALFSSRRPVDFDWVVLAVLGLWFLLPLGQDVSHVDLTGCALALGAGACWAIYILSGQRAGAEHGPATVAIGSLIAALIFVPIGALQAGEALWHWSVIPLGLAVAILSTALPYSLEMIALTRLPTRTFGTLMSMEPALAAVSGMIFLGETLTPIQLLALGAIIAASMGSTLTVRKESKIKELDIN

SEQ ID NO: 8 - DNA, 888 bp, synthetic construct
  source 1..888: mol_type = other DNA; note = RhtA V123D NT
atgcctggttcattacgtaaaatgccggtctggttaccaatagtcatattgctcgttgccatggcgtctattcagggtggagcctcgttagctaagtcactttttcctctggtgggcgcaccgggtgtcactgcgctgcgtctggcattaggaacgctgatcctcatcgcgttctttaagccatggcgactgcgctttgccaaagagcaacggttaccgctgttgttttacggcgtttcgctgggtgggatgaattatcttttttatctttctattcagacagtaccgctgggtattgcggtggcgctggagttcaccggaccactggcggtggcgctgttctcttctcgtcgcccggtagatttcgactgggttgtgctggcggttcttggtctgtggttcctgctaccgctggggcaagacgtttcccatgtcgatttaaccggctgtgcgctggcactgggggccggggcttgttgggctatttacattttaagtgggcaacgcgcaggagcggaacatggccctgcgacggtggcaattggttcgttgattgcagcgttaattttcgtgccaattggagcgcttcaggctggtgaagcactctggcactggtcggttattccattgggtctggctgtcgctattctctcgaccgctctgccttattcgctggaaatgattgccctcacccgtttgccaacacggacatttggtacgctgatgagcatggaaccggcgctggctgccgtttccgggatgattttcctcggagaaacactgacacccatacagctactggcgctcggcgctatcatcgccgcttcaatggggtctacgctgacagtacgcaaagagagcaaaataaaagaattagacattaattaa

SEQ ID NO: 9 - protein, 295 aa, synthetic construct
  source 1..295: note = RhtA V123E AA
MPGSLRKMPVWLPIVILLVAMASIQGGASLAKSLFPLVGAPGVTALRLALGTLILIAFFKPWRLRFAKEQRLPLLFYGVSLGGMNYLFYLSIQTVPLGIAVALEFTGPLAVALFSSRRPVDFEWVVLAVLGLWFLLPLGQDVSHVDLTGCALALGAGACWAIYILSGQRAGAEHGPATVAIGSLIAALIFVPIGALQAGEALWHWSVIPLGLAVAILSTALPYSLEMIALTRLPTRTFGTLMSMEPALAAVSGMIFLGETLTPIQLLALGAIIAASMGSTLTVRKESKIKELDIN

SEQ ID NO: 10 - DNA, 888 bp, synthetic construct
  source 1..888: mol_type = other DNA; note = RhtA V123E NT
atgcctggttcattacgtaaaatgccggtctggttaccaatagtcatattgctcgttgccatggcgtctattcagggtggagcctcgttagctaagtcactttttcctctggtgggcgcaccgggtgtcactgcgctgcgtctggcattaggaacgctgatcctcatcgcgttctttaagccatggcgactgcgctttgccaaagagcaacggttaccgctgttgttttacggcgtttcgctgggtgggatgaattatcttttttatctttctattcagacagtaccgctgggtattgcggtggcgctggagttcaccggaccactggcggtggcgctgttctcttctcgtcgcccggtagatttcgaatgggttgtgctggcggttcttggtctgtggttcctgctaccgctggggcaagacgtttcccatgtcgatttaaccggctgtgcgctggcactgggggccggggcttgttgggctatttacattttaagtgggcaacgcgcaggagcggaacatggccctgcgacggtggcaattggttcgttgattgcagcgttaattttcgtgccaattggagcgcttcaggctggtgaagcactctggcactggtcggttattccattgggtctggctgtcgctattctctcgaccgctctgccttattcgctggaaatgattgccctcacccgtttgccaacacggacatttggtacgctgatgagcatggaaccggcgctggctgccgtttccgggatgattttcctcggagaaacactgacacccatacagctactggcgctcggcgctatcatcgccgcttcaatggggtctacgctgacagtacgcaaagagagcaaaataaaagaattagacattaattaa

SEQ ID NO: 11 - protein, 295 aa, synthetic construct
  source 1..295: note = RhtA V123F AA
MPGSLRKMPVWLPIVILLVAMASIQGGASLAKSLFPLVGAPGVTALRLALGTLILIAFFKPWRLRFAKEQRLPLLFYGVSLGGMNYLFYLSIQTVPLGIAVALEFTGPLAVALFSSRRPVDFFWVVLAVLGLWFLLPLGQDVSHVDLTGCALALGAGACWAIYILSGQRAGAEHGPATVAIGSLIAALIFVPIGALQAGEALWHWSVIPLGLAVAILSTALPYSLEMIALTRLPTRTFGTLMSMEPALAAVSGMIFLGETLTPIQLLALGAIIAASMGSTLTVRKESKIKELDIN

SEQ ID NO: 12 - DNA, 888 bp, synthetic construct
  source 1..888: mol_type = other DNA; note = RhtA V123F NT
atgcctggttcattacgtaaaatgccggtctggttaccaatagtcatattgctcgttgccatggcgtctattcagggtggagcctcgttagctaagtcactttttcctctggtgggcgcaccgggtgtcactgcgctgcgtctggcattaggaacgctgatcctcatcgcgttctttaagccatggcgactgcgctttgccaaagagcaacggttaccgctgttgttttacggcgtttcgctgggtgggatgaattatcttttttatctttctattcagacagtaccgctgggtattgcggtggcgctggagttcaccggaccactggcggtggcgctgttctcttctcgtcgcccggtagatttcttctgggttgtgctggcggttcttggtctgtggttcctgctaccgctggggcaagacgtttcccatgtcgatttaaccggctgtgcgctggcactgggggccggggcttgttgggctatttacattttaagtgggcaacgcgcaggagcggaacatggccctgcgacggtggcaattggttcgttgattgcagcgttaattttcgtgccaattggagcgcttcaggctggtgaagcactctggcactggtcggttattccattgggtctggctgtcgctattctctcgaccgctctgccttattcgctggaaatgattgccctcacccgtttgccaacacggacatttggtacgctgatgagcatggaaccggcgctggctgccgtttccgggatgattttcctcggagaaacactgacacccatacagctactggcgctcggcgctatcatcgccgcttcaatggggtctacgctgacagtacgcaaagagagcaaaataaaagaattagacattaattaa

SEQ ID NO: 13 - protein, 295 aa, synthetic construct
  source 1..295: note = RhtA V123G AA
MPGSLRKMPVWLPIVILLVAMASIQGGASLAKSLFPLVGAPGVTALRLALGTLILIAFFKPWRLRFAKEQRLPLLFYGVSLGGMNYLFYLSIQTVPLGIAVALEFTGPLAVALFSSRRPVDFGWVVLAVLGLWFLLPLGQDVSHVDLTGCALALGAGACWAIYILSGQRAGAEHGPATVAIGSLIAALIFVPIGALQAGEALWHWSVIPLGLAVAILSTALPYSLEMIALTRLPTRTFGTLMSMEPALAAVSGMIFLGETLTPIQLLALGAIIAASMGSTLTVRKESKIKELDIN

SEQ ID NO: 14 - DNA, 888 bp, synthetic construct
  source 1..888: mol_type = other DNA; note = RhtA V123G NT
atgcctggttcattacgtaaaatgccggtctggttaccaatagtcatattgctcgttgccatggcgtctattcagggtggagcctcgttagctaagtcactttttcctctggtgggcgcaccgggtgtcactgcgctgcgtctggcattaggaacgctgatcctcatcgcgttctttaagccatggcgactgcgctttgccaaagagcaacggttaccgctgttgttttacggcgtttcgctgggtgggatgaattatcttttttatctttctattcagacagtaccgctgggtattgcggtggcgctggagttcaccggaccactggcggtggcgctgttctcttctcgtcgcccggtagatttcggctgggttgtgctggcggttcttggtctgtggttcctgctaccgctggggcaagacgtttcccatgtcgatttaaccggctgtgcgctggcactgggggccggggcttgttgggctatttacattttaagtgggcaacgcgcaggagcggaacatggccctgcgacggtggcaattggttcgttgattgcagcgttaattttcgtgccaattggagcgcttcaggctggtgaagcactctggcactggtcggttattccattgggtctggctgtcgctattctctcgaccgctctgccttattcgctggaaatgattgccctcacccgtttgccaacacggacatttggtacgctgatgagcatggaaccggcgctggctgccgtttccgggatgattttcctcggagaaacactgacacccatacagctactggcgctcggcgctatcatcgccgcttcaatggggtctacgctgacagtacgcaaagagagcaaaataaaagaattagacattaattaa

SEQ ID NO: 15 - protein, 295 aa, synthetic construct
  source 1..295: note = RhtA V123H AA
MPGSLRKMPVWLPIVILLVAMASIQGGASLAKSLFPLVGAPGVTALRLALGTLILIAFFKPWRLRFAKEQRLPLLFYGVSLGGMNYLFYLSIQTVPLGIAVALEFTGPLAVALFSSRRPVDHTWVVLAVLGLWFLLPLGQDVSHVDLTGCALALGAGACWAIYILSGQRAGAEHGPATVAIGSLIAALIFVPIGALQAGEALWHWSVIPLGLAVAILSTALPYSLEMIALTRLPTRTFGTLMSMEPALAAVSGMIFLGETLTPIQLLALGAIIAASMGSTLTVRKESKIKELDIN

SEQ ID NO: 16 - DNA, 888 bp, synthetic construct
  source 1..888: mol_type = other DNA; note = RhtA V123H NT
atgcctggttcattacgtaaaatgccggtctggttaccaatagtcatattgctcgttgccatggcgtctattcagggtggagcctcgttagctaagtcactttttcctctggtgggcgcaccgggtgtcactgcgctgcgtctggcattaggaacgctgatcctcatcgcgttctttaagccatggcgactgcgctttgccaaagagcaacggttaccgctgttgttttacggcgtttcgctgggtgggatgaattatcttttttatctttctattcagacagtaccgctgggtattgcggtggcgctggagttcaccggaccactggcggtggcgctgttctcttctcgtcgcccggtagatttccactgggttgtgctggcggttcttggtctgtggttcctgctaccgctggggcaagacgtttcccatgtcgatttaaccggctgtgcgctggcactgggggccggggcttgttgggctatttacattttaagtgggcaacgcgcaggagcggaacatggccctgcgacggtggcaattggttcgttgattgcagcgttaattttcgtgccaattggagcgcttcaggctggtgaagcactctggcactggtcggttattccattgggtctggctgtcgctattctctcgaccgctctgccttattcgctggaaatgattgccctcacccgtttgccaacacggacatttggtacgctgatgagcatggaaccggcgctggctgccgtttccgggatgattttcctcggagaaacactgacacccatacagctactggcgctcggcgctatcatcgccgcttcaatggggtctacgctgacagtacgcaaagagagcaaaataaaagaattagacattaattaa

SEQ ID NO: 17 - protein, 295 aa, synthetic construct
  source 1..295: note = RhtA V123I AA
MPGSLRKMPVWLPIVILLVAMASIQGGASLAKSLFPLVGAPGVTALRLALGTLILIAFFKPWRLRFAKEQRLPLLFYGVSLGGMNYLFYLSIQTVPLGIAVALEFTGPLAVALFSSRRPVDFIWVVLAVLGLWFLLPLGQDVSHVDLTGCALALGAGACWAIYILSGQRAGAEHGPATVAIGSLIAALIFVPIGALQAGEALWHWSVIPLGLAVAILSTALPYSLEMIALTRLPTRTFGTLMSMEPALAAVSGMIFLGETLTPIQLLALGAIIAASMGSTLTVRKESKIKELDIN

SEQ ID NO: 18 - DNA, 888 bp, synthetic construct
  source 1..888: mol_type = other DNA; note = RhtA V123I NT
atgcctggttcattacgtaaaatgccggtctggttaccaatagtcatattgctcgttgccatggcgtctattcagggtggagcctcgttagctaagtcactttttcctctggtgggcgcaccgggtgtcactgcgctgcgtctggcattaggaacgctgatcctcatcgcgttctttaagccatggcgactgcgctttgccaaagagcaacggttaccgctgttgttttacggcgtttcgctgggtgggatgaattatcttttttatctttctattcagacagtaccgctgggtattgcggtggcgctggagttcaccggaccactggcggtggcgctgttctcttctcgtcgcccggtagatttcatctgggttgtgctggcggttcttggtctgtggttcctgctaccgctggggcaagacgtttcccatgtcgatttaaccggctgtgcgctggcactgggggccggggcttgttgggctatttacattttaagtgggcaacgcgcaggagcggaacatggccctgcgacggtggcaattggttcgttgattgcagcgttaattttcgtgccaattggagcgcttcaggctggtgaagcactctggcactggtcggttattccattgggtctggctgtcgctattctctcgaccgctctgccttattcgctggaaatgattgccctcacccgtttgccaacacggacatttggtacgctgatgagcatggaaccggcgctggctgccgtttccgggatgattttcctcggagaaacactgacacccatacagctactggcgctcggcgctatcatcgccgcttcaatggggtctacgctgacagtacgcaaagagagcaaaataaaagaattagacattaattaa

SEQ ID NO: 19 - protein, 295 aa, synthetic construct
  source 1..295: note = RhtA V123K AA
MPGSLRKMPVWLPIVILLVAMASIQGGASLAKSLFPLVGAPGVTALRLALGTLILIAFFKPWRLRFAKEQRLPLLFYGVSLGGMNYLFYLSIQTVPLGIAVALEFTGPLAVALFSSRRPVDFKWVVLAVLGLWFLLPLGQDVSHVDLTGCALALGAGACWAIYILSGQRAGAEHGPATVAIGSLIAALIFVPIGALQAGEALWHWSVIPLGLAVAILSTALPYSLEMIALTRLPTRTFGTLMSMEPALAAVSGMIFLGETLTPIQLLALGAIIAASMGSTLTVRKESKIKELDIN

SEQ ID NO: 20 - DNA, 888 bp, synthetic construct
  source 1..888: mol_type = other DNA; note = RhtA V123K NT
atgcctggttcattacgtaaaatgccggtctggttaccaatagtcatattgctcgttgccatggcgtctattcagggtggagcctcgttagctaagtcactttttcctctggtgggcgcaccgggtgtcactgcgctgcgtctggcattaggaacgctgatcctcatcgcgttctttaagccatggcgactgcgctttgccaaagagcaacggttaccgctgttgttttacggcgtttcgctgggtgggatgaattatcttttttatctttctattcagacagtaccgctgggtattgcggtggcgctggagttcaccggaccactggcggtggcgctgttctcttctcgtcgcccggtagatttcaagtgggttgtgctggcggttcttggtctgtggttcctgctaccgctggggcaagacgtttcccatgtcgatttaaccggctgtgcgctggcactgggggccggggcttgttgggctatttacattttaagtgggcaacgcgcaggagcggaacatggccctgcgacggtggcaattggttcgttgattgcagcgttaattttcgtgccaattggagcgcttcaggctggtgaagcactctggcactggtcggttattccattgggtctggctgtcgctattctctcgaccgctctgccttattcgctggaaatgattgccctcacccgtttgccaacacggacatttggtacgctgatgagcatggaaccggcgctggctgccgtttccgggatgattttcctcggagaaacactgacacccatacagctactggcgctcggcgctatcatcgccgcttcaatggggtctacgctgacagtacgcaaagagagcaaaataaaagaattagacattaattaa

SEQ ID NO: 21 - protein, 295 aa, synthetic construct
  source 1..295: note = RhtA V123L AA
MPGSLRKMPVWLPIVILLVAMASIQGGASLAKSLFPLVGAPGVTALRLALGTLILIAFFKPWRLRFAKEQRLPLLFYGVSLGGMNYLFYLSIQTVPLGIAVALEFTGPLAVALFSSRRPVDFLWVVLAVLGLWFLLPLGQDVSHVDLTGCALALGAGACWAIYILSGQRAGAEHGPATVAIGSLIAALIFVPIGALQAGEALWHWSVIPLGLAVAILSTALPYSLEMIALTRLPTRTFGTLMSMEPALAAVSGMIFLGETLTPIQLLALGAIIAASMGSTLTVRKESKIKELDIN

SEQ ID NO: 22 - DNA, 888 bp, synthetic construct
  source 1..888: mol_type = other DNA; note = RhtA V123L NT
atgcctggttcattacgtaaaatgccggtctggttaccaatagtcatattgctcgttgccatggcgtctattcagggtggagcctcgttagctaagtcactttttcctctggtgggcgcaccgggtgtcactgcgctgcgtctggcattaggaacgctgatcctcatcgcgttctttaagccatggcgactgcgctttgccaaagagcaacggttaccgctgttgttttacggcgtttcgctgggtgggatgaattatcttttttatctttctattcagacagtaccgctgggtattgcggtggcgctggagttcaccggaccactggcggtggcgctgttctcttctcgtcgcccggtagatttcctctgggttgtgctggcggttcttggtctgtggttcctgctaccgctggggcaagacgtttcccatgtcgatttaaccggctgtgcgctggcactgggggccggggcttgttgggctatttacattttaagtgggcaacgcgcaggagcggaacatggccctgcgacggtggcaattggttcgttgattgcagcgttaattttcgtgccaattggagcgcttcaggctggtgaagcactctggcactggtcggttattccattgggtctggctgtcgctattctctcgaccgctctgccttattcgctggaaatgattgccctcacccgtttgccaacacggacatttggtacgctgatgagcatggaaccggcgctggctgccgtttccgggatgattttcctcggagaaacactgacacccatacagctactggcgctcggcgctatcatcgccgcttcaatggggtctacgctgacagtacgcaaagagagcaaaataaaagaattagacattaattaa

SEQ ID NO: 23 - protein, 295 aa, synthetic construct
  source 1..295: note = RhtA V123M AA
MPGSLRKMPVWLPIVILLVAMASIQGGASLAKSLFPLVGAPGVTALRLALGTLILIAFFKPWRLRFAKEQRLPLLFYGVSLGGMNYLFYLSIQTVPLGIAVALEFTGPLAVALFSSRRPVDFMWVVLAVLGLWFLLPLGQDVSHVDLTGCALALGAGACWAIYILSGQRAGAEHGPATVAIGSLIAALIFVPIGALQAGEALWHWSVIPLGLAVAILSTALPYSLEMIALTRLPTRTFGTLMSMEPALAAVSGMIFLGETLTPIQLLALGAIIAASMGSTLTVRKESKIKELDIN

SEQ ID NO: 24 - DNA, 888 bp, synthetic construct
  source 1..888: mol_type = other DNA; note = RhtA V123M NT
atgcctggttcattacgtaaaatgccggtctggttaccaatagtcatattgctcgttgccatggcgtctattcagggtggagcctcgttagctaagtcactttttcctctggtgggcgcaccgggtgtcactgcgctgcgtctggcattaggaacgctgatcctcatcgcgttctttaagccatggcgactgcgctttgccaaagagcaacggttaccgctgttgttttacggcgtttcgctgggtgggatgaattatcttttttatctttctattcagacagtaccgctgggtattgcggtggcgctggagttcaccggaccactggcggtggcgctgttctcttctcgtcgcccggtagatttcatgtgggttgtgctggcggttcttggtctgtggttcctgctaccgctggggcaagacgtttcccatgtcgatttaaccggctgtgcgctggcactgggggccggggcttgttgggctatttacattttaagtgggcaacgcgcaggagcggaacatggccctgcgacggtggcaattggttcgttgattgcagcgttaattttcgtgccaattggagcgcttcaggctggtgaagcactctggcactggtcggttattccattgggtctggctgtcgctattctctcgaccgctctgccttattcgctggaaatgattgccctcacccgtttgccaacacggacatttggtacgctgatgagcatggaaccggcgctggctgccgtttccgggatgattttcctcggagaaacactgacacccatacagctactggcgctcggcgctatcatcgccgcttcaatggggtctacgctgacagtacgcaaagagagcaaaataaaagaattagacattaattaa

SEQ ID NO: 25 - protein, 295 aa, synthetic construct
  source 1..295: note = RhtA V123N AA
MPGSLRKMPVWLPIVILLVAMASIQGGASLAKSLFPLVGAPGVTALRLALGTLILIAFFKPWRLRFAKEQRLPLLFYGVSLGGMNYLFYLSIQTVPLGIAVALEFTGPLAVALFSSRRPVDFNWVVLAVLGLWFLLPLGQDVSHVDLTGCALALGAGACWAIYILSGQRAGAEHGPATVAIGSLIAALIFVPIGALQAGEALWHWSVIPLGLAVAILSTALPYSLEMIALTRLPTRTFGTLMSMEPALAAVSGMIFLGETLTPIQLLALGAIIAASMGSTLTVRKESKIKELDIN

SEQ ID NO: 26 - DNA, 888 bp, synthetic construct
  source 1..888: mol_type = other DNA; note = RhtA V123N NT
atgcctggttcattacgtaaaatgccggtctggttaccaatagtcatattgctcgttgccatggcgtctattcagggtggagcctcgttagctaagtcactttttcctctggtgggcgcaccgggtgtcactgcgctgcgtctggcattaggaacgctgatcctcatcgcgttctttaagccatggcgactgcgctttgccaaagagcaacggttaccgctgttgttttacggcgtttcgctgggtgggatgaattatcttttttatctttctattcagacagtaccgctgggtattgcggtggcgctggagttcaccggaccactggcggtggcgctgttctcttctcgtcgcccggtagatttcaactgggttgtgctggcggttcttggtctgtggttcctgctaccgctggggcaagacgtttcccatgtcgatttaaccggctgtgcgctggcactgggggccggggcttgttgggctatttacattttaagtgggcaacgcgcaggagcggaacatggccctgcgacggtggcaattggttcgttgattgcagcgttaattttcgtgccaattggagcgcttcaggctggtgaagcactctggcactggtcggttattccattgggtctggctgtcgctattctctcgaccgctctgccttattcgctggaaatgattgccctcacccgtttgccaacacggacatttggtacgctgatgagcatggaaccggcgctggctgccgtttccgggatgattttcctcggagaaacactgacacccatacagctactggcgctcggcgctatcatcgccgcttcaatggggtctacgctgacagtacgcaaagagagcaaaataaaagaattagacattaattaa

SEQ ID NO: 27 - protein, 295 aa, synthetic construct
  source 1..295: note = RhtA V123P AA
MPGSLRKMPVWLPIVILLVAMASIQGGASLAKSLFPLVGAPGVTALRLALGTLILIAFFKPWRLRFAKEQRLPLLFYGVSLGGMNYLFYLSIQTVPLGIAVALEFTGPLAVALFSSRRPVDFPWVVLAVLGLWFLLPLGQDVSHVDLTGCALALGAGACWAIYILSGQRAGAEHGPATVAIGSLIAALIFVPIGALQAGEALWHWSVIPLGLAVAILSTALPYSLEMIALTRLPTRTFGTLMSMEPALAAVSGMIFLGETLTPIQLLALGAIIAASMGSTLTVRKESKIKELDIN

SEQ ID NO: 28 - DNA, 888 bp, synthetic construct
  source 1..888: mol_type = other DNA; note = RhtA V123P NT
atgcctggttcattacgtaaaatgccggtctggttaccaatagtcatattgctcgttgccatggcgtctattcagggtggagcctcgttagctaagtcactttttcctctggtgggcgcaccgggtgtcactgcgctgcgtctggcattaggaacgctgatcctcatcgcgttctttaagccatggcgactgcgctttgccaaagagcaacggttaccgctgttgttttacggcgtttcgctgggtgggatgaattatcttttttatctttctattcagacagtaccgctgggtattgcggtggcgctggagttcaccggaccactggcggtggcgctgttctcttctcgtcgcccggtagatttcccatgggttgtgctggcggttcttggtctgtggttcctgctaccgctggggcaagacgtttcccatgtcgatttaaccggctgtgcgctggcactgggggccggggcttgttgggctatttacattttaagtgggcaacgcgcaggagcggaacatggccctgcgacggtggcaattggttcgttgattgcagcgttaattttcgtgccaattggagcgcttcaggctggtgaagcactctggcactggtcggttattccattgggtctggctgtcgctattctctcgaccgctctgccttattcgctggaaatgattgccctcacccgtttgccaacacggacatttggtacgctgatgagcatggaaccggcgctggctgccgtttccgggatgattttcctcggagaaacactgacacccatacagctactggcgctcggcgctatcatcgccgcttcaatggggtctacgctgacagtacgcaaagagagcaaaataaaagaattagacattaattaa

SEQ ID NO: 29 - protein, 295 aa, synthetic construct
  source 1..295: note = RhtA V123Q AA
MPGSLRKMPVWLPIVILLVAMASIQGGASLAKSLFPLVGAPGVTALRLALGTLILIAFFKPWRLRFAKEQRLPLLFYGVSLGGMNYLFYLSIQTVPLGIAVALEFTGPLAVALFSSRRPVDFQWVVLAVLGLWFLLPLGQDVSHVDLTGCALALGAGACWAIYILSGQRAGAEHGPATVAIGSLIAALIFVPIGALQAGEALWHWSVIPLGLAVAILSTALPYSLEMIALTRLPTRTFGTLMSMEPALAAVSGMIFLGETLTPIQLLALGAIIAASMGSTLTVRKESKIKELDIN

SEQ ID NO: 30 - DNA, 888 bp, synthetic construct
  source 1..888: mol_type = other DNA
atgcctggttcattacgtaaaatgccggtctggttaccaatagtcatattgctcgttgccatggcgtctattcagggtggagcctcgttagctaagtcactttttcctctggtgggcgcaccgggtgtcactgcgctgcgtctggcattaggaacgctgatcctcatcgcgttctttaagccatggcgactgcgctttgccaaagagcaacggttaccgctgttgttttacggcgtttcgctgggtgggatgaattatcttttttatctttctattcagacagtaccgctgggtattgcggtggcgctggagttcaccggaccactggcggtggcgctgttctcttctcgtcgcccggtagatttccagtgggttgtgctggcggttcttggtctgtggttcctgctaccgctggggcaagacgtttcccatgtcgatttaaccggctgtgcgctggcactgggggccggggcttgttgggctatttacattttaagtgggcaacgcgcaggagcggaacatggccctgcgacggtggcaattggttcgttgattgcagcgttaattttcgtgccaattggagcgcttcaggctggtgaagcactctggcactggtcggttattccattgggtctggctgtcgctattctctcgaccgctctgccttattcgctggaaatgattgccctcacccgtttgccaacacggacatttggtacgctgatgagcatggaaccggcgctggctgccgtttccgggatgattttcctcggagaaacactgacacccatacagctactggcgctcggcgctatcatcgccgcttcaatggggtctacgctgacagtacgcaaagagagcaaaataaaagaattagacattaattaa

SEQ ID NO: 31 - protein, 295 aa, synthetic construct
  source 1..295: note = RhtA V123R AA
MPGSLRKMPVWLPIVILLVAMASIQGGASLAKSLFPLVGAPGVTALRLALGTLILIAFFKPWRLRFAKEQRLPLLFYGVSLGGMNYLFYLSIQTVPLGIAVALEFTGPLAVALFSSRRPVDFRWVVLAVLGLWFLLPLGQDVSHVDLTGCALALGAGACWAIYILSGQRAGAEHGPATVAIGSLIAALIFVPIGALQAGEALWHWSVIPLGLAVAILSTALPYSLEMIALTRLPTRTFGTLMSMEPALAAVSGMIFLGETLTPIQLLALGAIIAASMGSTLTVRKESKIKELDIN

SEQ ID NO: 32 - DNA, 888 bp, synthetic construct
  source 1..888: mol_type = other DNA; note = RhtA V123R NT
atgcctggttcattacgtaaaatgccggtctggttaccaatagtcatattgctcgttgccatggcgtctattcagggtggagcctcgttagctaagtcactttttcctctggtgggcgcaccgggtgtcactgcgctgcgtctggcattaggaacgctgatcctcatcgcgttctttaagccatggcgactgcgctttgccaaagagcaacggttaccgctgttgttttacggcgtttcgctgggtgggatgaattatcttttttatctttctattcagacagtaccgctgggtattgcggtggcgctggagttcaccggaccactggcggtggcgctgttctcttctcgtcgcccggtagatttccgctgggttgtgctggcggttcttggtctgtggttcctgctaccgctggggcaagacgtttcccatgtcgatttaaccggctgtgcgctggcactgggggccggggcttgttgggctatttacattttaagtgggcaacgcgcaggagcggaacatggccctgcgacggtggcaattggttcgttgattgcagcgttaattttcgtgccaattggagcgcttcaggctggtgaagcactctggcactggtcggttattccattgggtctggctgtcgctattctctcgaccgctctgccttattcgctggaaatgattgccctcacccgtttgccaacacggacatttggtacgctgatgagcatggaaccggcgctggctgccgtttccgggatgattttcctcggagaaacactgacacccatacagctactggcgctcggcgctatcatcgccgcttcaatggggtctacgctgacagtacgcaaagagagcaaaataaaagaattagacattaattaa

SEQ ID NO: 33 - protein, 295 aa, synthetic construct
  source 1..295: note = RhtA V123S AA
MPGSLRKMPVWLPIVILLVAMASIQGGASLAKSLFPLVGAPGVTALRLALGTLILIAFFKPWRLRFAKEQRLPLLFYGVSLGGMNYLFYLSIQTVPLGIAVALEFTGPLAVALFSSRRPVDFSWVVLAVLGLWFLLPLGQDVSHVDLTGCALALGAGACWAIYILSGQRAGAEHGPATVAIGSLIAALIFVPIGALQAGEALWHWSVIPLGLAVAILSTALPYSLEMIALTRLPTRTFGTLMSMEPALAAVSGMIFLGETLTPIQLLALGAIIAASMGSTLTVRKESKIKELDIN

SEQ ID NO: 34 - DNA, 888 bp, synthetic construct
  source 1..888: mol_type = other DNA; note = RhtA V123S NT
atgcctggttcattacgtaaaatgccggtctggttaccaatagtcatattgctcgttgccatggcgtctattcagggtggagcctcgttagctaagtcactttttcctctggtgggcgcaccgggtgtcactgcgctgcgtctggcattaggaacgctgatcctcatcgcgttctttaagccatggcgactgcgctttgccaaagagcaacggttaccgctgttgttttacggcgtttcgctgggtgggatgaattatcttttttatctttctattcagacagtaccgctgggtattgcggtggcgctggagttcaccggaccactggcggtggcgctgttctcttctcgtcgcccggtagatttctcctgggttgtgctggcggttcttggtctgtggttcctgctaccgctggggcaagacgtttcccatgtcgatttaaccggctgtgcgctggcactgggggccggggcttgttgggctatttacattttaagtgggcaacgcgcaggagcggaacatggccctgcgacggtggcaattggttcgttgattgcagcgttaattttcgtgccaattggagcgcttcaggctggtgaagcactctggcactggtcggttattccattgggtctggctgtcgctattctctcgaccgctctgccttattcgctggaaatgattgccctcacccgtttgccaacacggacatttggtacgctgatgagcatggaaccggcgctggctgccgtttccgggatgattttcctcggagaaacactgacacccatacagctactggcgctcggcgctatcatcgccgcttcaatggggtctacgctgacagtacgcaaagagagcaaaataaaagaattagacattaattaa

SEQ ID NO: 35 - protein, 295 aa, synthetic construct
  source 1..295: note = RhtA V123T AA
MPGSLRKMPVWLPIVILLVAMASIQGGASLAKSLFPLVGAPGVTALRLALGTLILIAFFKPWRLRFAKEQRLPLLFYGVSLGGMNYLFYLSIQTVPLGIAVALEFTGPLAVALFSSRRPVDFTWVVLAVLGLWFLLPLGQDVSHVDLTGCALALGAGACWAIYILSGQRAGAEHGPATVAIGSLIAALIFVPIGALQAGEALWHWSVIPLGLAVAILSTALPYSLEMIALTRLPTRTFGTLMSMEPALAAVSGMIFLGETLTPIQLLALGAIIAASMGSTLTVRKESKIKELDIN

SEQ ID NO: 36 - DNA, 888 bp, synthetic construct; identical to SEQ ID NO: 2
  source 1..888: mol_type = other DNA; note = RhtA V123T NT

SEQ ID NO: 37 - protein, 295 aa, synthetic construct
  source 1..295: note = RhtA V123W AA
MPGSLRKMPVWLPIVILLVAMASIQGGASLAKSLFPLVGAPGVTALRLALGTLILIAFFKPWRLRFAKEQRLPLLFYGVSLGGMNYLFYLSIQTVPLGIAVALEFTGPLAVALFSSRRPVDFWWVVLAVLGLWFLLPLGQDVSHVDLTGCALALGAGACWAIYILSGQRAGAEHGPATVAIGSLIAALIFVPIGALQAGEALWHWSVIPLGLAVAILSTALPYSLEMIALTRLPTRTFGTLMSMEPALAAVSGMIFLGETLTPIQLLALGAIIAASMGSTLTVRKESKIKELDIN

SEQ ID NO: 38 - DNA, 888 bp, synthetic construct
  source 1..888: mol_type = other DNA; note = RhtA V123W NT
atgcctggttcattacgtaaaatgccggtctggttaccaatagtcatattgctcgttgccatggcgtctattcagggtggagcctcgttagctaagtcactttttcctctggtgggcgcaccgggtgtcactgcgctgcgtctggcattaggaacgctgatcctcatcgcgttctttaagccatggcgactgcgctttgccaaagagcaacggttaccgctgttgttttacggcgtttcgctgggtgggatgaattatcttttttatctttctattcagacagtaccgctgggtattgcggtggcgctggagttcaccggaccactggcggtggcgctgttctcttctcgtcgcccggtagatttctggtgggttgtgctggcggttcttggtctgtggttcctgctaccgctggggcaagacgtttcccatgtcgatttaaccggctgtgcgctggcactgggggccggggcttgttgggctatttacattttaagtgggcaacgcgcaggagcggaacatggccctgcgacggtggcaattggttcgttgattgcagcgttaattttcgtgccaattggagcgcttcaggctggtgaagcactctggcactggtcggttattccattgggtctggctgtcgctattctctcgaccgctctgccttattcgctggaaatgattgccctcacccgtttgccaacacggacatttggtacgctgatgagcatggaaccggcgctggctgccgtttccgggatgattttcctcggagaaacactgacacccatacagctactggcgctcggcgctatcatcgccgcttcaatggggtctacgctgacagtacgcaaagagagcaaaataaaagaattagacattaattaa

SEQ ID NO: 39 - protein, 295 aa, synthetic construct
  source 1..295: note = RhtA V123Y AA
MPGSLRKMPVWLPIVILLVAMASIQGGASLAKSLFPLVGAPGVTALRLALGTLILIAFFKPWRLRFAKEQRLPLLFYGVSLGGMNYLFYLSIQTVPLGIAVALEFTGPLAVALFSSRRPVDFYWVVLAVLGLWFLLPLGQDVSHVDLTGCALALGAGACWAIYILSGQRAGAEHGPATVAIGSLIAALIFVPIGALQAGEALWHWSVIPLGLAVAILSTALPYSLEMIALTRLPTRTFGTLMSMEPALAAVSGMIFLGETLTPIQLLALGAIIAASMGSTLTVRKESKIKELDIN

SEQ ID NO: 40 - DNA, 888 bp, synthetic construct
  source 1..888: mol_type = other DNA; note = RhtA V123Y NT
atgcctggttcattacgtaaaatgccggtctggttaccaatagtcatattgctcgttgccatggcgtctattcagggtggagcctcgttagctaagtcactttttcctctggtgggcgcaccgggtgtcactgcgctgcgtctggcattaggaacgctgatcctcatcgcgttctttaagccatggcgactgcgctttgccaaagagcaacggttaccgctgttgttttacggcgtttcgctgggtgggatgaattatcttttttatctttctattcagacagtaccgctgggtattgcggtggcgctggagttcaccggaccactggcggtggcgctgttctcttctcgtcgcccggtagatttctactgggttgtgctggcggttcttggtctgtggttcctgctaccgctggggcaagacgtttcccatgtcgatttaaccggctgtgcgctggcactgggggccggggcttgttgggctatttacattttaagtgggcaacgcgcaggagcggaacatggccctgcgacggtggcaattggttcgttgattgcagcgttaattttcgtgccaattggagcgcttcaggctggtgaagcactctggcactggtcggttattccattgggtctggctgtcgctattctctcgaccgctctgccttattcgctggaaatgattgccctcacccgtttgccaacacggacatttggtacgctgatgagcatggaaccggcgctggctgccgtttccgggatgattttcctcggagaaacactgacacccatacagctactggcgctcggcgctatcatcgccgcttcaatggggtctacgctgacagtacgcaaagagagcaaaataaaagaattagacattaattaa

SEQ ID NO: 41 - DNA, 38 bp, synthetic construct
  source 1..38: mol_type = other DNA; note = rhtA F
agacacaccgggagttcatcatgcctggttcattacgt

SEQ ID NO: 42 - DNA, 37 bp, synthetic construct
  source 1..37: mol_type = other DNA; note = rhtA R
aattcgagctcggtacccttaattaatgtctaattct

SEQ ID NO: 43 - DNA, 38 bp, synthetic construct
  source 1..38: mol_type = other DNA; note = PrhtB F
gtcgactctagaggatcccccgggtaatctgcctctta

SEQ ID NO: 44 - DNA, 38 bp, synthetic construct
  source 1..38: mol_type = other DNA; note = PrhtB R
acgtaatgaaccaggcatgatgaactcccggtgtgtct

SEQ ID NO: 45 - DNA, 35 bp, synthetic construct
  source 1..35: mol_type = other DNA; note = rhtBC up F
gctgcaggaattcgatccgccagatcatcaacata

SEQ ID NO: 46 - DNA, 36 bp, synthetic construct
  source 1..36: mol_type = other DNA; note = rhtBC up R
ttttttgtctctcgatatccccagccaaatcaagta

SEQ ID NO: 47 - DNA, 36 bp, synthetic construct
  source 1..36: mol_type = other DNA; note = rhtBC down F
acttgatttggctggggatatcgagagacaaaaaag

SEQ ID NO: 48 - DNA, 34 bp, synthetic construct
  source 1..34: mol_type = other DNA; note = rhtBC down R
aggtcgactagcgtgataggagccgtgcgggaac

SEQ ID NO: 49 - DNA, 37 bp, synthetic construct
  source 1..37: mol_type = other DNA; note = rhtA up F
tgcaggaattcgataaagaaccgatcacacccagcgg

SEQ ID NO: 50 - DNA, 36 bp, synthetic construct
  source 1..36: mol_type = other DNA; note = rhtA up R
agagcggtcgagagaatagatatctcctttctccca

SEQ ID NO: 51 - DNA, 36 bp, synthetic construct
  source 1..36: mol_type = other DNA; note = rhtA down F
tgggagaaaggagatatctattctctcgaccgctct

SEQ ID NO: 52 - DNA, 35 bp, synthetic construct
  source 1..35: mol_type = other DNA; note = rhtA down R
agctaggtcgactagcgtgatggctatgtgttccg

SEQ ID NO: 53 - DNA, 19 bp, synthetic construct
  source 1..19: mol_type = other DNA; note = rhtABC up F
gatttaactaatttagcgg

SEQ ID NO: 54 - DNA, 19 bp, synthetic construct
  source 1..19: mol_type = other DNA; note = rhtABC up R
ccgcttctaatcactttgg

SEQ ID NO: 55 - DNA, 19 bp, synthetic construct
  source 1..19: mol_type = other DNA; note = rhtABC down F
ggctgaacctcctgctgcc

SEQ ID NO: 56 - DNA, 19 bp, synthetic construct
  source 1..19: mol_type = other DNA; note = rhtABC down R
cagcaataccagacgacgg

SEQ ID NO: 57 - DNA, 35 bp, synthetic construct
  source 1..35: mol_type = other DNA; note = Ncgl0998 up F
cgagctcggtaccctaataattctgcttcccgacg

SEQ ID NO: 58 - DNA, 30 bp, synthetic construct
  source 1..30: mol_type = other DNA; note = Ncgl0998 up R
ccacaaattaagggacggtcgatgtcgagg

SEQ ID NO: 59 - DNA, 35 bp, synthetic construct
  source 1..35: mol_type = other DNA; note = PgapA F
ctcgacatcgaccgtcccttaatttgtggattcac

SEQ ID NO: 60 - DNA, 34 bp, synthetic construct
  source 1..34: mol_type = other DNA; note = PgapA R
cgtaatgaaccaggcatgttgtgtctcctctaaa

SEQ ID NO: 61 - DNA, 35 bp, synthetic construct
  source 1..35: mol_type = other DNA; note = rhtA_m F
ttagaggagacacaacatgcctggttcattacgta

SEQ ID NO: 62 - DNA, 35 bp, synthetic construct
  source 1..35: mol_type = other DNA; note = rhtA_m R
tcgggctcttccggttcccttaattaatgtctaat

SEQ ID NO: 63 - DNA, 35 bp, synthetic construct
  source 1..35: mol_type = other DNA; note = Ncgl0998 dn F
agacattaattaagggaaccggaagagcccgattg

SEQ ID NO: 64 - DNA, 38 bp, synthetic construct
  source 1..38: mol_type = other DNA; note = Ncgl0998 dn R
tagaggatccccgaaaaggaagaagtctgagaagaagg

SEQ ID NO: 65 - DNA, 35 bp, synthetic construct
  source 1..35: mol_type = other DNA; note = up F
tcgagctcggtaccctgtctccgtatgcagtgagc

SEQ ID NO: 66 - DNA, 30 bp, synthetic construct
  source 1..30: mol_type = other DNA; note = up R
ggatgtttctttggagcttcgctcaatcat

SEQ ID NO: 67 - DNA, 35 bp, synthetic construct
  source 1..35: mol_type = other DNA; note = hom F
tataggagaacaatcatgacctcagcatctgcccc

SEQ ID NO: 68 - DNA, 22 bp, synthetic construct
  source 1..22: mol_type = other DNA; note = G378E R
gccaaaacctccacgcgatctt

SEQ ID NO: 69 - DNA, 22 bp, synthetic construct
  source 1..22: mol_type = other DNA; note = G378E F
aagatcgcgtggaggttttggc

SEQ ID NO: 70 - DNA, 25 bp, synthetic construct
  source 1..25: mol_type = other DNA; note = R398Q R
gcgctcttcctgttggattgtacgc

SEQ ID NO: 71 - DNA, 25 bp, synthetic construct
  source 1..25: mol_type = other DNA; note = R398Q F
gcgtacaatccaacaggaagagcgc

SEQ ID NO: 72 - DNA, 35 bp, synthetic construct
  source 1..35: mol_type = other DNA; note = hom R
ctctagaggatccccgactgcggaatgttgttgtg

SEQ ID NO: 73 - DNA, 20 bp, synthetic construct
  source 1..20: mol_type = other DNA; note = hom conf F
tgggtaggtcgagttgttaa

SEQ ID NO: 74 - DNA, 20 bp, synthetic construct
  source 1..20: mol_type = other DNA; note = hom conf R
cagcgcagtcgcacgaatat

SEQ ID NO: 75 - DNA, 35 bp, synthetic construct
  source 1..35: mol_type = other DNA; note = lysC promoter Up 1
tcgagctcggtacccgacaggacaagcactggttg

SEQ ID NO: 76 - DNA, 35 bp, synthetic construct
  source 1..35: mol_type = other DNA; note = lysC promoter Up 2
agtagcgctgggatgtttctctttgtgcacctttc

SEQ ID NO: 77 - DNA, 30 bp, synthetic construct
  source 1..30: mol_type = other DNA; note = lysC Down 1
gaacatcgaaaagatttccacctctgagat

SEQ ID NO: 78 - DNA, 35 bp, synthetic construct
  source 1..35: mol_type = other DNA; note = lysC Down 2
ctctagaggatccccgttcacctcagagacgatta

SEQ ID NO: 79 - DNA, 35 bp, synthetic construct
  source 1..35: mol_type = other DNA; note = lysC 1
cgaaaggaaacactcatggccctggtcgtacagaa

SEQ ID NO: 80 - DNA, 30 bp, synthetic construct
  source 1..30: mol_type = other DNA; note = lysC 2
ggtggaaatcttttcgatgttcacgttgac

SEQ ID NO: 81 - DNA, 20 bp, synthetic construct
  source 1..20: mol_type = other DNA; note = confirm lysC 1
acattccacccattactgca

SEQ ID NO: 82 - DNA, 20 bp, synthetic construct
  source 1..20: mol_type = other DNA; note = confirm lysC 2
tcttcatcggtttcgaaggt

SEQ ID NO: 83 - DNA, 20 bp, synthetic construct
  source 1..20: mol_type = other DNA; note = outside F
cacgtgcagattcggtctcg

SEQ ID NO: 84 - DNA, 20 bp, synthetic construct
  source 1..20: mol_type = other DNA; note = outside R
ttcggttcttcaacgtctgg

SEQ ID NO: 85 - DNA, 35 bp, synthetic construct
  source 1..35: mol_type = other DNA; note = pDCM2-PgapA_rhtA V123A F
cgtcgcccggtagatttcgcctgggttgtgctggc

SEQ ID NO: 86 - DNA, 20 bp, synthetic construct
  source 1..20: mol_type = other DNA; note = pDCM2-PgapA_rhtA V123A R
gaaatctaccgggcgacgag

SEQ ID NO: 87 - DNA, 35 bp, synthetic construct
  source 1..35: mol_type = other DNA; note = pDCM2-PgapA_rhtA V123C F
cgtcgcccggtagatttctgctgggttgtgctggc

SEQ ID NO: 88 - DNA, 20 bp, synthetic construct
  source 1..20: mol_type = other DNA; note = pDCM2-PgapA_rhtA V123C R
gaaatctaccgggcgacgag

SEQ ID NO: 89 - DNA, 35 bp, synthetic construct
  source 1..35: mol_type = other DNA; note = pDCM2-PgapA_rhtA V123D F
cgtcgcccggtagatttcgactgggttgtgctggc

SEQ ID NO: 90 - DNA, 20 bp, synthetic construct
  source 1..20: mol_type = other DNA; note = pDCM2-PgapA_rhtA V123D R
gaaatctaccgggcgacgag

SEQ ID NO: 91 - DNA, 35 bp, synthetic construct
  source 1..35: mol_type = other DNA; note = pDCM2-PgapA_rhtA V123E F
cgtcgcccggtagatttcgaatgggttgtgctggc

SEQ ID NO: 92 - DNA, 20 bp, synthetic construct
  source 1..20: mol_type = other DNA; note = pDCM2-PgapA_rhtA V123E R
gaaatctaccgggcgacgag

SEQ ID NO: 93 - DNA, 35 bp, synthetic construct
  source 1..35: mol_type = other DNA; note = pDCM2-PgapA_rhtA V123F F
cgtcgcccggtagatttcttctgggttgtgctggc

SEQ ID NO: 94 - DNA, 20 bp, synthetic construct
  source 1..20: mol_type = other DNA; note = pDCM2-PgapA_rhtA V123F R
gaaatctaccgggcgacgag

SEQ ID NO: 95 - DNA, 35 bp, synthetic construct
  source 1..35: mol_type = other DNA; note = pDCM2-PgapA_rhtA V123G F
cgtcgcccggtagatttcggctgggttgtgctggc

SEQ ID NO: 96 - DNA, 20 bp, synthetic construct
  source 1..20: mol_type = other DNA; note = pDCM2-PgapA_rhtA V123G R
gaaatctaccgggcgacgag

SEQ ID NO: 97 - DNA, 35 bp, synthetic construct
  source 1..35: mol_type = other DNA; note = pDCM2-PgapA_rhtA V123H F
cgtcgcccggtagatttccactgggttgtgctggc

SEQ ID NO: 98 - DNA, 20 bp, synthetic construct
  source 1..20: mol_type = other DNA; note = pDCM2-PgapA_rhtA V123H R
gaaatctaccgggcgacgag

SEQ ID NO: 99 - DNA, 35 bp, synthetic construct
  source 1..35: mol_type = other DNA; note = pDCM2-PgapA_rhtA V123I F
cgtcgcccggtagatttcatctgggttgtgctggc

SEQ ID NO: 100 - DNA, 20 bp, synthetic construct
  source 1..20: mol_type = other DNA; note = pDCM2-PgapA_rhtA V123I R
gaaatctaccgggcgacgag

SEQ ID NO: 101 - DNA, 35 bp, synthetic construct
  source 1..35: mol_type = other DNA; note = pDCM2-PgapA_rhtA V123K F
cgtcgcccggtagatttcaagtgggttgtgctggc

SEQ ID NO: 102 - DNA, 20 bp, synthetic construct
  source 1..20: mol_type = other DNA; note = pDCM2-PgapA_rhtA V123K R
gaaatctaccgggcgacgag

SEQ ID NO: 103 - DNA, 35 bp, synthetic construct
  source 1..35: mol_type = other DNA; note = pDCM2-PgapA_rhtA V123L F
cgtcgcccggtagatttcctctgggttgtgctggc

SEQ ID NO: 104 - DNA, 20 bp, synthetic construct
  source 1..20: mol_type = other DNA; note = pDCM2-PgapA_rhtA V123L R
gaaatctaccgggcgacgag

SEQ ID NO: 105 - DNA, 35 bp, synthetic construct
  source 1..35: mol_type = other DNA; note = pDCM2-PgapA_rhtA V123M F
cgtcgcccggtagatttcatgtgggttgtgctggc

SEQ ID NO: 106 - DNA, 20 bp, synthetic construct
  source 1..20: mol_type = other DNA; note = pDCM2-PgapA_rhtA V123M R
gaaatctaccgggcgacgag

SEQ ID NO: 107 - DNA, 35 bp, synthetic construct
  source 1..35: mol_type = other DNA; note = pDCM2-PgapA_rhtA V123N F
cgtcgcccggtagatttcaactgggttgtgctggc

SEQ ID NO: 108 - DNA, 20 bp, synthetic construct
  source 1..20: mol_type = other DNA; note = pDCM2-PgapA_rhtA V123N R
gaaatctaccgggcgacgag

SEQ ID NO: 109 - DNA, 35 bp, synthetic construct
  source 1..35: mol_type = other DNA; note = pDCM2-PgapA_rhtA V123P F
cgtcgcccggtagatttcccatgggttgtgctggc

SEQ ID NO: 110 - DNA, 20 bp, synthetic construct
  source 1..20: mol_type = other DNA; note = pDCM2-PgapA_rhtA V123P R
gaaatctaccgggcgacgag

SEQ ID NO: 111 - DNA, 35 bp, synthetic construct
  source 1..35: mol_type = other DNA; note = pDCM2-PgapA_rhtA V123Q F
cgtcgcccggtagatttccagtgggttgtgctggc

SEQ ID NO: 112 - DNA, 20 bp, synthetic construct
  source 1..20: mol_type = other DNA; note = pDCM2-PgapA_rhtA V123Q R
gaaatctaccgggcgacgag

SEQ ID NO: 113 - DNA, 35 bp, synthetic construct
  source 1..35: mol_type = other DNA; note = pDCM2-PgapA_rhtA V123R F
cgtcgcccggtagatttccgctgggttgtgctggc

SEQ ID NO: 114 - DNA, 20 bp, synthetic construct
  source 1..20: mol_type = other DNA; note = pDCM2-PgapA_rhtA V123R R
gaaatctaccgggcgacgag

SEQ ID NO: 115 - DNA, 35 bp, synthetic construct
  source 1..35: mol_type = other DNA; note = pDCM2-PgapA_rhtA V123S F
cgtcgcccggtagatttctcctgggttgtgctggc

SEQ ID NO: 116 - DNA, 20 bp, synthetic construct
  source 1..20: mol_type = other DNA; note = pDCM2-PgapA_rhtA V123S R
gaaatctaccgggcgacgag

SEQ ID NO: 117 - DNA, 35 bp, synthetic construct
  source 1..35: mol_type = other DNA; note = pDCM2-PgapA_rhtA V123T F
cgtcgcccggtagatttcacctgggttgtgctggc

SEQ ID NO: 118 - DNA, 20 bp, synthetic construct
  source 1..20: mol_type = other DNA; note = pDCM2-PgapA_rhtA V123T R
gaaatctaccgggcgacgag

SEQ ID NO: 119 - DNA, 35 bp, synthetic construct
  source 1..35: mol_type = other DNA; note = pDCM2-PgapA_rhtA V123W F
cgtcgcccggtagatttctggtgggttgtgctggc

SEQ ID NO: 120 - DNA, 20 bp, synthetic construct
  source 1..20: mol_type = other DNA; note = pDCM2-PgapA_rhtA V123W R
gaaatctaccgggcgacgag

SEQ ID NO: 121 - DNA, 35 bp, synthetic construct
  source 1..35: mol_type = other DNA; note = pDCM2-PgapA_rhtA V123Y F
cgtcgcccggtagatttctactgggttgtgctggc

SEQ ID NO: 122 - DNA, 20 bp, synthetic construct
  source 1..20: mol_type = other DNA; note = pDCM2-PgapA_rhtA V123Y R
gaaatctaccgggcgacgag